European Patent Specification EP 3 935 152 B1, published November 8, 2023. Title: induced photoreceptor cells. Applicant: Technische Unversität Dresden. The sequence listing filed with the application follows.

SEQUENCE LISTING (13 sequences)

SEQ ID NO: 1 - protein, 1098 aa, Homo sapiens [sequence omitted]

SEQ ID NO: 2 - protein, 2241 aa, Homo sapiens
  human GON4L isoform A, GenBank: AAR01260.1
MLPCKKRRTTVTESLQHKGNQEENNVDLESAVKPESDQVKDLSSVSLSWDPSHGRVAGFEVQSLQDAGNQLGMEDTSLSSGMLTQNTNVPILEGVDVAISQGITLPSLESFHPLNIHIGKGKLHATGSKRGKKMTLRPGPVTQEDRCDHLTLKEPFSGEPSEEVKEEGGKPQMNSEGEIPSLPSGSQSAKPVSQPRKSTQPDVCASPQEKPLRTLFHQPEEEIEDGGLFIPMEEQDNEESEKRRKKKKGTKRKRDGRGQEGTLAYDLKLDDMLDRTLEDGAKQHNLTAVNVRNILHEVITNEHVVAMMKAAISETEDMPMFEPKMTRSKLKEVVEKGVVIPTWNISPIKKANEIKPPQFVDIHLEEDDSSDEEYQPDDEEEDETAEESLLESDVESTASSPRGAKKSRLRQSSEMTETDEESGILSEAEKVTTPAIRHISAEVVPMGPPPPPKPKQTRDSTFMEKLHAVDEELASSPVCMDSFQPMDDSLIAFRTRSKMPLKDVPLGQLEAELQAPDITPDMYDPNTADDEDWKMWLGGLMNDDVGNEDEADDDDDPEYNFLEDLDEPDTEDFRTDRAVRITKKEVNELMEELFETFQDEMGFSNMEDDGPEEEECVAEPRPNFNTPQALRFEEPLANLLNEQHRTVKELFEQLKMKKSSAKQLQEVEKVKPQSEKVHQTLILDPAQRKRLQQQMQQHVQLLTQIHLLATCNPNLNPEATTTRIFLKELGTFAQSSIALHHQYNPKFQTLFQPCNLMGAMQLIEDFSTHVSIDCSPHKTVKKTANEFPCLPKQVAWILATSKVFMYPELLPVCSLKAKNPQDKIVFTKAEDNLLALGLKHFEGTEFPNPLISKYLLTCKTAHQLTVRIKNLNMNRAPDNIIKFYKKTKQLPVLGKCCEEIQPHQWKPPIEREEHRLPFWLKASLPSIQEELRHMADGAREVGNMTGTTEINSDRSLEKDNLELGSESRYPLLLPKGVVLKLKPVATRFPRKAWRQKRSSVLKPLLIQPSPSLQPSFNPGKTPARSTHSEAPPSKMVLRIPHPIQPATVLQTVPGVPPLGVSGGESFESPAALPAVPPEARTSFPLSESQTLLSSAPVPKVMLPSLAPSKFRKPYVRRRPSKRRGVKASPCMKPAPVIHHPASVIFTVPATTVKIVSLGGGCNMIQPVNAAVAQSPQTIPITTLLVNPTSFPCPLNQSLVASSVSPLIVSGNSVNLPIPSTPEDKAHVNVDIACAVADGENAFQGLEPKLEPQELSPLSATVFPKVEHSPGPPLADAECQEGLSENSACRWTVVKTEEGRQALEPLPQGIQESLNNPTPGDLEEIVKMEPEEAREEISGSPERDICDDIKVEHAVELDTGAPSEELSSAGEVTKQTVLQKEEERSQPTKTPSSSQEPPDEGTSGTDVNKGSSKNALSSMDPEVRLSSPPGKPEDSSSVDGQSVGTPVGPETGGEKNGPEEEEEEDFDDLTQDEEDEMSSASEESVLSVPELQETMEKLTWLASERRMSQEGESEEENSQEENSEPEEEEEEEAEGMESLQKEDEMTDEAVGDSAEKPPTFASPETAPEVETSRTPPGESIKAAGKGRNNHRARNKRGSRARASKDTSKLLLLYDEDILERDPLREQKDLAFAQAYLTRVREALQHIPGKYEDFLQVIYEFESSTQRRTAVDLYKSLQILLQDWPQLLKDFAAFLLPEQALACGLFEEQQAFEKSRKFLRQLEICFAENPSHHQKIIKVLQGCADCLPQEITELKTQMWQLLKGHDHLQDEFSIFFDHLRPAASRMGDFEEINWTEEKEYEFDGFEEVALPDVEEEEEPPKIPTASKNKRKKEIGVQNHDKETEWPDGAKDCACSCHEGGPDSKLKKSKRRSCSHCSSKVCDSKSYKSKEPHELVGSSPHREASPMPGAKEAGQGKDMMEEEAPEERESTEATQSRTVRTTRKGEMPVSAGLAVGSTLPSPREVTVTERLLLDGPPPHSPETPQFPPTTGAVLYTVKRNQVGPEVRSCPKASPRLQKEREGQKAVSESEALMLVWDASETEKLPGTVEPPASFLSPVSSKTRDAGRRHVSGKPDTQERWLPSSRARVKTRDRTCPVHESPSGIDTSETSPKAPRGGLAKDSGTQAKGPEGEQQPKAAEATVCANNSKVSSTGEKVVLWTREADRVILTMCQEQGAQPQTFNIISQQLGNKTPAEVSHRFRELMQLFHTACEASSEDEDDATSTSNADQLSDHGDLLSEEELDE

SEQ ID NO: 3 - protein, 1529 aa, Homo sapiens
  human GON4L isoform B, GenBank: AAR01262.1
MLPCKKRRTTVTESLQHKGNQEENNVDLESAVKPESDQVKDLSSVSLSWDPSHGRVAGFEVQSLQDAGNQLGMEDTSLSSGMLTQNTNVPILEGVDVAISQGITLPSLESFHPLNIHIGKGKLHATGSKRGKKMTLRPGPVTQEDRCDHLTLKEPFSGEPSEEVKEEGGKPQMNSEGEIPSLPSGSQSAKPVSQPRKSTQPDVCASPQEKPLRTLFHQPEEEIEDGGLFIPMEEQDNEESEKRRKKKKGTKRKRDGRGQEGTLAYDLKLDDMLDRTLEDGAKQHNLTAVNVRNILHEVITNEHVVAMMKAAISETEDMPMFEPKMTRSKLKEVVEKGVVIPTWNISPIKKANEIKPPQFVDIHLEEDDSSDEEYQPDDEEEDETAEESLLESDVESTASSPRGAKKSRLRQSSEMTETDEESGILSEAEKVTAPAIRHISAEVVPMGPPPPPKPKQTRDSTFMEKLHAVDEELASSPVCMDSFQPMDDSLIAFRTRSKMPLKDVPLGQLEAELQAPDITPDMYDPNTADDEDWKMWLGGLMNDDVGNEDEADDDDDPEYNFLEDLDEPDTEDFRTDRAVRITKKEVNELMEELFETFQDEMGFSNMEDDGPEEEECVAEPRPNFNTPQALRFEEPLANLLNEQHRTVKELFEQLKMKKSSAKQLQEVEKVKPQSEKVHQTLILDPAQRKRLQQQMQQHVQLLTQIHLLATCNPNLNPEATTTRIFLKELGTFAQSSIALHHQYNPKFQTLFQPCNLMGAMQLIEDFSTHVSIDCSPHKTVKKTANEFPCLPKQVAWILATSKVFMYPELLPVCSLKAKNPQDKIVFTKAEDNLLALGLKHFEGTEFPNPLISKYLLTCKTAHQLTVRIKNLNMNRAPDNIIKFYKKTKQLPVLGKCCEEIQPHQWKPPIEREEHRLPFWLKASLPSIQEELRHMADGAREVGNMTGTTEINSDRSLEKDNLELGSESRYPLLLPKGVVLKLKPVATRSPRKAWRQKRSSVLKPLLIQPSPSLQPSFNPGKTPARSTHSEAPPSKMVLRIPHPIQPATVLQTVPGVPPLGVSGGESFESPAALPAVPPEARTSFPLSESQTLLSSAPVPKVMLPSLAPSKFRKPYVRRRPSKRRGVKASPCMKPAPVIHHPASVIFTVPATTVKIVSLGGGCNMIQPVNAAVAQSPQTIPITTLLVNPTSFPCPLNQSLVASSVSPLIVSGNSVNLPIPSTPEDKAHVNVDIACAVADGENAFQGLEPKLEPQELSPLSATVFPKVEHSPGPPLADAECQEGLSENSACRWTVVKTEEGRQALEPLPQGIQESLNNPTPGDLEEIVKMEPEEAREEISGSPERDICDDIKVEHAVELDTGAPSEELSSAGEVTKQTVLQKEEGRSQPTKTPSSSQEPPDEGTSGTDVNKGSSKNALSSMDPEVRLSSPPGKPEDSSSVDGQSVGTPVGPETGGEKNGPEEEEEEDFDDLTQDEEDEMSSASEESVLSVPELQVRAGEYSQVFRGLSNMYHLLICHLLACCTMDSPKIICI

SEQ ID NO: 4 - protein, 2241 aa, Homo sapiens; identical to SEQ ID NO: 2
  human GON4L isoform C, GenBank: AAR01261.1

SEQ ID NO: 5 - protein, 356 aa, Homo sapiens
  human NEUROD1, GenBank: BAJ84018.1
MTKSYSESGLMGEPQPQGPPSWTDECLSSQDEEHEADKKEDDLEAMNAEEDSLRNGGEEEDEDEDLEEEEEEEEEDDDQKPKRRGPKKKKMTKARLERFKLRRMKANARERNRMHGLNAALDNLRKVVPCYSKTQKLSKIETLRLAKNYIWALSEILRSGKSPDLVSFVQTLCKGLSQPTTNLVAGCLQLNPRTFLPEQNQDMPPHLPTASASFPVHPYSYQSPGLPSPPYGTMDSSHVFHVKPPPHAYSAALEPFFESPLTDCTSPSFDGPLSPPLSINGNFSFKHEPSAEFEKNYAFTMHYPAATLAGAQSHGSIFSGTAAPRCEIPIDNIMSFDSHSHHERVMSAQLNAIFHD

SEQ ID NO: 6 - protein, 297 aa, Homo sapiens
  human OTX2 Isoform A, NCBI Reference Sequence: NP_068374.1
MMSYLKQPPYAVNGLSLTTSGMDLLHPSVGYPGPWASCPAATPRKQRRERTTFTRAQLDVLEALFAKTRYPDIFMREEVALKINLPESRVQVWFKNRRAKCRQQQQQQQNGGQNKVRPAKKKTSPAREVSSESGTSGQFTPPSSTSVPTIASSSAPVSIWSPASISPLSDPLSTSSSCMQRSYPMTYTQASGYSQGYAGSTSYFGGMDCGSYLTPMHHQLPGPGATLSPMGTNAVTSHLNQSPASLSTQGYGASSLGFNSTTDCLDYKDQTASWKLNFNADCLDYKDQTSSWKFQVL

SEQ ID NO: 7 - protein, 289 aa, Homo sapiens
  human OTX2 Isoform B, NCBI Reference Sequence: NP_001257453.1
MMSYLKQPPYAVNGLSLTTSGMDLLHPSVGYPATPRKQRRERTTFTRAQLDVLEALFAKTRYPDIFMREEVALKINLPESRVQVWFKNRRAKCRQQQQQQQNGGQNKVRPAKKKTSPAREVSSESGTSGQFTPPSSTSVPTIASSSAPVSIWSPASISPLSDPLSTSSSCMQRSYPMTYTQASGYSQGYAGSTSYFGGMDCGSYLTPMHHQLPGPGATLSPMGTNAVTSHLNQSPASLSTQGYGASSLGFNSTTDCLDYKDQTASWKLNFNADCLDYKDQTSSWKFQVL

SEQ ID NO: 8 - DNA, 4587 bp, Homo sapiens
atgttgccctgtaagaagagaagaactacagtgacagagtccctacagcataaaggcaatcaagaggaaaacaacgtagacctagaatcagccgttaaaccagaatctgaccaggttaaggacttgagttcggtgtcactatcctgggatccaagtcatggcagagtagctggcttcgaagtacagtctttgcaggatgcaggaaatcagcttggtatggaggatacatctctgagctctggaatgctcacccagaacacaaatgtaccaattctagaaggtgttgatgtggccatctctcagggaatcaccctaccttccttggagtcttttcacccccttaatatacacattggtaaaggaaaactccacgctactggctcaaagagagggaaaaaaatgacactcaggcctgggccagttacccaagaagacagatgtgatcatcttaccctaaaggagcctttttcaggagagcctagtgaagaagtcaaggaagaaggagggaaacctcaaatgaattctgaaggggagataccttccctgccatcaggcagccaatctgcaaaaccagtaagccagcccaggaaatcaacccagccagatgtttgtgcctctcctcaagaaaagccactcaggactctgtttcaccaacctgaggaagagatagaagatggtggactcttcattccaatggaagaacaagacaatgaagaaagtgagaaaaggagaaaaaagaaaaagggtaccaagaggaaacgagatggaaggggtcaagaagggaccttggcatatgacctgaaactggatgacatgcttgaccgtaccttggaggatggtgccaagcagcacaatctaacagcagtcaatgtccgaaacatccttcatgaagtaatcacaaatgaacacgtggtagctatgatgaaagcagccatcagtgagacggaagatatgccaatgtttgagcctaaaatgacacgctctaaactgaaggaagtagtggaaaaaggagtggtaattccaacatggaatatttcaccaattaagaaggccaatgaaattaagcctcctcagtttgtggatatccaccttgaagaagatgattcctcagatgaagaataccagccggatgatgaagaagaagatgaaactgctgaagagagcttattggaaagtgatgttgaaagcactgcttcatctccacgtggggcaaagaaatccagattgaggcagtcttctgagatgactgaaacagatgaggagagtggcatattatcagaggctgagaaagtcaccacaccagccatcaggcacatcagtgctgaggtagtgcccatggggcccccgccccctccaaagccgaaacagaccagagatagtactttcatggagaagttacatgcggtagatgaggagctggcttccagtccagtctgcatggattctttccagcccatggatgacagtctcattgcatttcgaacgcgttctaagatgcccctgaaagatgttcccctgggccaattagaggcagagctccaagctccagacatcactccagatatgtatgaccccaatacggcagatgatgaggactggaagatgtggctggggggacttatgaatgatgatgtggggaatgaagatgaagcagatgatgatgatgatccagaatataatttcctggaagacctcgatgaaccagacacagaggatttccggactgaccgggcagtgagaatcaccaaaaaggaagtaaatgagctgatggaagagctgtttgaaactttccaagatgagatgggattctccaacatggaagatgatggcccagaagaggaggagtgtgtagctgagcctcgtcctaactttaacacccctcaagctctacggtttgaggaaccactggccaacctgttaaatgaacaacatcggacagtgaaggagctatttgaacagctgaagatgaagaaatcttcagccaaacagctgcaggaagtagagaaggttaaaccccagagtgagaaagttcatcagactctgattctggacccagcacagaggaagagactccagcagcagatgcagcagcacgttcagctcttgacccaaatccaccttcttgccacctgcaaccccaacctcaatccggaggccactaccaccaggatatttcttaaagagctgggaacctttgctcaaagctccatcgcccttcaccatcagtacaaccccaagtttcagaccctgttccaaccctgtaacttgatgggagctatgcagctgattgaagacttcagcacacatgtcagcattgactgcagccctcataaaactgtcaagaagactgcgaatgaatttccctgtttgccaaagcaagtggcttggattctggccacaagcaaggttttcatgtatccagagttacttccagtgtgttccctgaaggcaaagaatccccaggataagatcgtcttcaccaaggctgaggacaatttgttagctttaggactgaagcattttgaaggaactgagtttcctaatcctctaatcagcaagtaccttctaacctgcaaaactgcccaccaactgacagtgagaatcaagaacctcaacatgaacagagctcctgacaacatcattaaattttataagaagaccaaacagctgccagtcctaggaaaatgctgtgaagagatccagccacatcagtggaagccacctatagagagagaagaacaccggctcccattctggttaaaggccagtctgccatccatccaggaagaactgcggcacatggctgatggtgctagagaggtaggaaatatgactggaaccactgagatcaactcagatcgaagcctagaaaaagacaatttggagttggggagtgaatctcggtacccactgctattgcctaagggtgtagtcctgaaactgaagccagttgccacccgtttccccaggaaggcttggagacagaagcgttcatcagtcctgaagcccctccttatccaacccagcccctctctccagcccagcttcaaccctgggaaaacaccagcccgatcaactcattcagaagcccctccgagcaaaatggtgctccggattcctcacccaatacagccagccactgttttacagacagttccaggtgtccctccactgggggtcagtggaggtgagagttttgagtctcctgcagcactgcctgctgtgccccctgaggccaggacaagcttccctctgtctgagtcccagactttgctctcttctgcccctgtgcccaaggtaatgctgccctcccttgccccttctaagtttcgaaagccatatgtgagacggagaccctcaaagagaagaggagtcaaggcctctccctgtatgaaacctgcccctgttatccaccaccctgcatctgttatcttcactgttcctgctaccactgtgaagattgtgagccttggcggtggctgtaacatgatccagcctgtcaatgcggctgtggcccagagtccccagactattcccatcactaccctcttggttaaccctacttccttcccctgtccattgaaccagtcccttgtggcctcctctgtctcacccttaattgtttctggcaattctgtgaatcttcctataccatccacccctgaagataaggcccacgtgaatgtggacattgcttgtgctgtggctgatggggaaaatgcctttcagggcctagaacccaaattagagccccaggaactatctcctctctctgctactgttttcccgaaagtggaacatagcccagggcctccactagcagatgcagagtgccaagaaggattgtcagagaatagtgcctgtcgctggaccgttgtgaaaacagaggaggggaggcaagctctggagccgctccctcagggcatccaggagtctctaaacaaccctacccctggggatttagaggaaattgtcaagatggaacctgaagaagctagagaggaaatcagtggatcccctgagcgtgatatttgtgatgacatcaaagtggaacatgctgtggaattggacactggtgccccaagcgaggagttgagcagtgctggagaagtaacgaaacagacagtcttacagaaggaagaggagaggagtcagccaactaaaaccccttcatcttctcaagagccccctgatgaaggaacctcagggacagatgtgaacaaaggatcatcaaagaatgctttgtcctcaatggatcctgaagtgaggcttagtagccccccagggaagccagaagattcatccagtgttgatggtcagtcagtggggactccagttgggccagaaactggaggagagaagaatgggccagaagaagaggaagaagaggactttgatgacctcacccaagatgaggaagatgaaatgtcatcagcttctgaggaatctgtgctttctgtcccagaactccaggtgagagctggagaatattctcaagtatttcgtggactcagtaatatgtatcacttattgatatgccacctgcttgcttgctgcactatggatagtcctaaaatcatttgtatt

SEQ ID NO: 9 - DNA, 4641 bp, Homo sapiens
atgttgccctgtaagaagagaagaactacagtgacagagtccctacagcataaaggcaatcaagaggaaaacaacgtagacctagaatcagccgttaaaccagaatctgaccaggttaaggacttgagttcggtgtcactatcctgggatccaagtcatggcagagtagctggcttcgaagtacagtctttgcaggatgcaggaaatcagcttggtatggaggatacatctctgagctctggaatgctcacccagaacacaaatgtaccaattctagaaggtgttgatgtggccatctctcagggaatcaccctaccttccttggagtcttttcacccccttaatatacacattggtaaaggaaaactccacgctactggctcaaagagagggaaaaaaatgacactcaggcctgggccagttacccaagaagacagatgtgatcatcttaccctaaaggagcctttttcaggagagcctagtgaagaagtcaaggaagaaggagggaaacctcaaatgaattctgaaggggagataccttccctgccatcaggcagccaatctgcaaaaccagtaagccagcccaggaaatcaacccagccagatgtttgtgcctctcctcaagaaaagccactcaggactctgtttcaccaacctgaggaagagatagaagatggtggactcttcattccaatggaagaacaagacaatgaagaaagtgagaaaaggagaaaaaagaaaaagggtaccaagaggaaacgagatggaaggggtcaagaagggaccttggcatatgacctgaaactggatgacatgcttgaccgtaccttggaggatggtgccaagcagcacaatctaacagcagtcaatgtccgaaacatccttcatgaagtaatcacaaatgaacacgtggtagctatgatgaaagcagccatcagtgagacggaagatatgccaatgtttgagcctaaaatgacacgctctaaactgaaggaagtagtggaaaaaggagtggtaattccaacatggaatatttcaccaattaagaaggccaatgaaattaagcctcctcagtttgtggatatccaccttgaagaagatgattcctcagatgaagaataccagccggatgatgaagaagaagatgaaactgctgaagagagcttattggaaagtgatgttgaaagcactgcttcatctccacgtggggcaaagaaatccagattgaggcagtcttctgagatgactgaaacagatgaggagagtggcatattatcagaggctgagaaagtcaccacaccagccatcaggcacatcagtgctgaggtagtgcccatggggcccccgccccctccaaagccgaaacagaccagagatagtactttcatggagaagttacatgcggtagatgaggagctggcttccagtccagtctgcatggattctttccagcccatggatgacagtctcattgcatttcgaacgcgttctaagatgcccctgaaagatgttcccctgggccaattagaggcagagctccaagctccagacatcactccagatatgtatgaccccaatacggcagatgatgaggactggaagatgtggctggggggacttatgaatgatgatgtggggaatgaagatgaagcagatgatgatgatgatccagaatataatttcctggaagacctcgatgaaccagacacagaggatttccggactgaccgggcagtgagaatcaccaaaaaggaagtaaatgagctgatggaagagctgtttgaaactttccaagatgagatgggattctccaacatggaagatgatggcccagaagaggaggagtgtgtagctgagcctcgtcctaactttaacacccctcaagctctacggtttgaggaaccactggccaacctgttaaatgaacaacatcggacagtgaaggagctatttgaacagctgaagatgaagaaatcttcagccaaacagctgcaggaagtagagaaggttaaaccccagagtgagaaagttcatcagactctgattctggacccagcacagaggaagagactccagcagcagatgcagcagcacgttcagctcttgacccaaatccaccttcttgccacctgcaaccccaacctcaatccggaggccactaccaccaggatatttcttaaagagctgggaacctttgctcaaagctccatcgcccttcaccatcagtacaaccccaagtttcagaccctgttccaaccctgtaacttgatgggagctatgcagctgattgaagacttcagcacacatgtcagcattgactgcagccctcataaaactgtcaagaagactgcgaatgaatttccctgtttgccaaagcaagtggcttggattctggccacaagcaaggttttcatgtatccagagttacttccagtgtgttccctgaaggcaaagaatccccaggataagatcgtcttcaccaaggctgaggacaatttgttagctttaggactgaagcattttgaaggaactgagtttcctaatcctctaatcagcaagtaccttctaacctgcaaaactgcccaccaactgacagtgagaatcaagaacctcaacatgaacagagctcctgacaacatcattaaattttataagaagaccaaacagctgccagtcctaggaaaatgctgtgaagagatccagccacatcagtggaagccacctatagagagagaagaacaccggctcccattctggttaaaggccagtctgccatccatccaggaagaactgcggcacatggctgatggtgctagagaggtaggaaatatgactggaaccactgagatcaactcagatcgaagcctagaaaaagacaatttggagttggggagtgaatctcggtacccactgctattgcctaagggtgtagtcctgaaactgaagccagttgccacccgtttccccaggaaggcttggagacagaagcgttcatcagtcctgaagcccctccttatccaacccagcccctctctccagcccagcttcaaccctgggaaaacaccagcccgatcaactcattcagaagcccctccgagcaaaatggtgctccggattcctcacccaatacagccagccactgttttacagacagttccaggtgtccctccactgggggtcagtggaggtgagagttttgagtctcctgcagcactgcctgctgtgccccctgaggccaggacaagcttccctctgtctgagtcccagactttgctctcttctgcccctgtgcccaaggtaatgctgccctcccttgccccttctaagtttcgaaagccatatgtgagacggagaccctcaaagagaagaggagtcaaggcctctccctgtatgaaacctgcccctgttatccaccaccctgcatctgttatcttcactgttcctgctaccactgtgaagattgtgagccttggcggtggctgtaacatgatccagcctgtcaatgcggctgtggcccagagtccccagactattcccatcactaccctcttggttaaccctacttccttcccctgtccattgaaccagtcccttgtggcctcctctgtctcacccttaattgtttctggcaattctgtgaatcttcctataccatccacccctgaagataaggcccacgtgaatgtggacattgcttgtgctgtggctgatggggaaaatgcctttcagggcctagaacccaaattagagccccaggaactatctcctctctctgctactgttttcccgaaagtggaacatagcccagggcctccactagcagatgcagagtgccaagaaggattgtcagagaatagtgcctgtcgctggaccgttgtgaaaacagaggaggggaggcaagctctggagccgctccctcagggcatccaggagtctctaaacaaccctacccctggggatttagaggaaattgtcaagatggaacctgaagaagctagagaggaaatcagtggatcccctgagcgtgatatttgtgatgacatcaaagtggaacatgctgtggaattggacactggtgccccaagcgaggagttgagcagtgctggagaagtaacgaaacagacagtcttacagaaggaagaggagaggagtcagccaactaaaaccccttcatcttctcaagagccccctgatgaaggaacctcagggacagatgtgaacaaaggatcatcaaagaatgctttgtcctcaatggatcctgaagtgaggcttagtagccccccagggaagccagaagattcatccagtgttgatggtcagtcagtggggactccagttgggccagaaactggaggagagaagaatgggccagaagaagaggaagaagaggactttgatgacctcacccaagatgaggaagatgaaatgtcatcagcttctgaggaatctgtgctttctgtcccagaactccaggtgagagctggagaatattctcaagtatttcgtggactcagtaatatgtatcacttattgatatgccacctgcttgcttgctgcactatggatagtcctaaaatcatttgtattctcgagggtaagcctatccctaaccctctcctcggtctcgattctacgtaatga

SEQ ID NO: 10 - DNA, 1068 bp, Homo sapiens
atgaccaaatcgtacagcgagagtgggctgatgggcgagcctcagccccaaggtcctccaagctggacagacgagtgtctcagttctcaggacgaggagcacgaggcagacaagaaggaggacgacctcgaagccatgaacgcagaggaggactcactgaggaacgggggagaggaggaggacgaagatgaggacctggaagaggaggaagaagaggaagaggaggatgacgatcaaaagcccaagagacgcggccccaaaaagaagaagatgactaaggctcgcctggagcgttttaaattgagacgcatgaaggctaacgcccgggagcggaaccgcatgcacggactgaacgcggcgctagacaacctgcgcaaggtggtgccttgctattctaagacgcagaagctgtccaaaatcgagactctgcgcttggccaagaactacatctgggctctgtcggagatcctgcgctcaggcaaaagcccagacctggtctccttcgttcagacgctttgcaagggcttatcccaacccaccaccaacctggttgcgggctgcctgcaactcaatcctcggacttttctgcctgagcagaaccaggacatgcccccccacctgccgacggccagcgcttccttccctgtacacccctactcctaccagtcgcctgggctgcccagtccgccttacggtaccatggacagctcccatgtcttccacgttaagcctccgccgcacgcctacagcgcagcgctggagcccttctttgaaagccctctgactgattgcaccagcccttcctttgatggacccctcagcccgccgctcagcatcaatggcaacttctctttcaaacacgaaccgtccgccgagtttgagaaaaattatgcctttaccatgcactatcctgcagcgacactggcaggggcccaaagccacggatcaatcttctcaggcaccgctgcccctcgctgcgagatccccatagacaatattatgtccttcgatagccattcacatcatgagcgagtcatgagtgcccagctcaatgccatatttcatgat

SEQ ID NO: 11 - DNA, 1122 bp, Homo sapiens
atgaccaaatcgtacagcgagagtgggctgatgggcgagcctcagccccaaggtcctccaagctggacagacgagtgtctcagttctcaggacgaggagcacgaggcagacaagaaggaggacgacctcgaagccatgaacgcagaggaggactcactgaggaacgggggagaggaggaggacgaagatgaggacctggaagaggaggaagaagaggaagaggaggatgacgatcaaaagcccaagagacgcggccccaaaaagaagaagatgactaaggctcgcctggagcgttttaaattgagacgcatgaaggctaacgcccgggagcggaaccgcatgcacggactgaacgcggcgctagacaacctgcgcaaggtggtgccttgctattctaagacgcagaagctgtccaaaatcgagactctgcgcttggccaagaactacatctgggctctgtcggagatcctgcgctcaggcaaaagcccagacctggtctccttcgttcagacgctttgcaagggcttatcccaacccaccaccaacctggttgcgggctgcctgcaactcaatcctcggacttttctgcctgagcagaaccaggacatgcccccccacctgccgacggccagcgcttccttccctgtacacccctactcctaccagtcgcctgggctgcccagtccgccttacggtaccatggacagctcccatgtcttccacgttaagcctccgccgcacgcctacagcgcagcgctggagcccttctttgaaagccctctgactgattgcaccagcccttcctttgatggacccctcagcccgccgctcagcatcaatggcaacttctctttcaaacacgaaccgtccgccgagtttgagaaaaattatgcctttaccatgcactatcctgcagcgacactggcaggggcccaaagccacggatcaatcttctcaggcaccgctgcccctcgctgcgagatccccatagacaatattatgtccttcgatagccattcacatcatgagcgagtcatgagtgcccagctcaatgccatatttcatgatctcgagggtaagcctatccctaaccctctcctcggtctcgattctacgtaatga

SEQ ID NO: 12 - DNA, 891 bp, Homo sapiens
atgatgtcttatcttaagcaaccgccttacgcagtcaatgggctgagtctgaccacttcgggtatggacttgctgcacccctccgtgggctacccggggccctgggcttcttgtcccgcagccaccccccggaaacagcgccgggagaggacgacgttcactcgggcgcagctagatgtgctggaagcactgtttgccaagacccggtacccagacatcttcatgcgagaggaggtggcactgaaaatcaacttgcccgagtcgagggtgcaggtatggtttaagaatcgaagagctaagtgccgccaacaacagcaacaacagcagaatggaggtcaaaacaaagtgagacctgccaaaaagaagacatctccagctcgggaagtgagttcagagagtggaacaagtggccaattcactcccccctctagcacctcagtcccgaccattgccagcagcagtgctcctgtgtctatctggagcccagcttccatctccccactgtcagatcccttgtccacctcctcttcctgcatgcagaggtcctatcccatgacctatactcaggcttcaggttatagtcaaggatatgctggctcaacttcctactttgggggcatggactgtggatcatatttgacccctatgcatcaccagcttcccggaccaggggccacactcagtcccatgggtaccaatgcagtcaccagccatctcaatcagtccccagcttctctttccacccagggatatggagcttcaagcttgggttttaactcaaccactgattgcttggattataaggaccaaactgcctcctggaagcttaacttcaatgctgactgcttggattataaagatcagacatcctcgtggaaattccaggttttg

SEQ ID NO: 13 - DNA, 945 bp, Homo sapiens
atgatgtcttatcttaagcaaccgccttacgcagtcaatgggctgagtctgaccacttcgggtatggacttgctgcacccctccgtgggctacccggggccctgggcttcttgtcccgcagccaccccccggaaacagcgccgggagaggacgacgttcactcgggcgcagctagatgtgctggaagcactgtttgccaagacccggtacccagacatcttcatgcgagaggaggtggcactgaaaatcaacttgcccgagtcgagggtgcaggtatggtttaagaatcgaagagctaagtgccgccaacaacagcaacaacagcagaatggaggtcaaaacaaagtgagacctgccaaaaagaagacatctccagctcgggaagtgagttcagagagtggaacaagtggccaattcactcccccctctagcacctcagtcccgaccattgccagcagcagtgctcctgtgtctatctggagcccagcttccatctccccactgtcagatcccttgtccacctcctcttcctgcatgcagaggtcctatcccatgacctatactcaggcttcaggttatagtcaaggatatgctggctcaacttcctactttgggggcatggactgtggatcatatttgacccctatgcatcaccagcttcccggaccaggggccacactcagtcccatgggtaccaatgcagtcaccagccatctcaatcagtccccagcttctctttccacccagggatatggagcttcaagcttgggttttaactcaaccactgattgcttggattataaggaccaaactgcctcctggaagcttaacttcaatgctgactgcttggattataaagatcagacatcctcgtggaaattccaggttttgctcgagggtaagcctatccctaaccctctcctcggtctcgattctacgtaatga